European Patent Application EP 4 722 381 A1, published April 8, 2026. Title: 一种基于5'连接的单链DNA特异的高通量测序方法. Applicant: 中国医学科学院基础医学研究所. The sequence listing filed with the application follows.

SEQUENCE LISTING (7 sequences)

SEQ ID NO: 1 - skipped

SEQ ID NO: 2 - DNA, 78 bp, synthetic construct
  source 1..78: mol_type = other DNA
gagatacccgtgnnnnnntaggtgcctacgaggagatacnnnnnnnnnngccgtaaggacgacttgggtaggcaccta

SEQ ID NO: 3 - skipped

SEQ ID NO: 4 - DNA, 78 bp, synthetic construct
  source 1..78: mol_type = other DNA
aatgatacggcgaccaccgagatctacactctttccctacacgacgctcttccgatcttaggtgcctacgaggagata

SEQ ID NO: 5 - DNA, 89 bp, synthetic construct
  source 1..89: mol_type = other DNA
caagcagaagacggcatacgagatcgtgatgtgactggagttcagacgtgtgctcttccgatcttttttttttttttttttttttttvn

SEQ ID NO: 6 - DNA, 89 bp, synthetic construct
  source 1..89: mol_type = other DNA
caagcagaagacggcatacgagatacatcggtgactggagttcagacgtgtgctcttccgatcttttttttttttttttttttttttvn

SEQ ID NO: 7 - DNA, 89 bp, synthetic construct
  source 1..89: mol_type = other DNA
caagcagaagacggcatacgagatgcctaagtgactggagttcagacgtgtgctcttccgatcttttttttttttttttttttttttvn